European Patent Application EP 4 692 107 A1, published February 11, 2026. Title: PEPTIDE HAVING SKIN CONDITION IMPROVEMENT ACTIVITY AND USES THEREOF. Applicant: CAREGEN CO., LTD. Application WO. The sequence listing filed with the application follows.

SEQUENCE LISTING (1 sequence)

SEQ ID NO: 1 - protein, 10 aa, synthetic construct
AERRREKCRC